European Patent Specification EP 3 778 650 B1, published August 20, 2025. Title: Fluorescent sensor for branched chain amino acid and uses thereof. Applicant: EAST CHINA UNIVERSITY OF SCIENCE AND TECHNOLOGY. The sequence listing filed with the application follows.

SEQUENCE LISTING (33 sequences)

SEQ ID NO: 1 - protein, 345 aa, Escherichia coli
  LivJ
MEDIKVAVVGAMSGPVAQYGDQEFTGAEQAVADINAKGGIKGNKLQIVKYDDACDPKQAVAVANKVVNDGIKYVIGHLCSSSTQPASDIYEDEGILMITPAATAPELTARGYQLILRTTGLDSDQGPTAAKYILEKVKPQRIAIVHDKQQYGEGLARAVQDGLKKGNANVVFFDGITAGEKDFSTLVARLKKENIDFVYYGGYHPEMGQILRQARAAGLKTQFMGPEGVANVSLSNIAGESAEGLLVTKPKNYDQVPANKPIVDAIKAKKQDPSGAFVWTTYAALQSLQAGLNQSDDPAEIAKYLKANSVDTVMGPLTWDEKGDLKGFEFGVFDWHANGTATDAK

SEQ ID NO: 2 - protein, 347 aa, Escherichia coli
  LivK
MDDIKVAVVGAMSGPIAQWGDMEFNGARQAIKDINAKGGIKGDKLVGVEYDDACDPKQAVAVANKIVNDGIKYVIGHLCSSSTQPASDIYEDEGILMISPGATNPELTQRGYQHIMRTAGLDSSQGPTAAKYILETVKPQRIAIIHDKQQYGEGLARSVQDGLKAANANVVFFDGITAGEKDFSALIARLKKENIDFVYYGGYYPEMGQMLRQARSVGLKTQFMGPEGVGNASLSNIAGDAAEGMLVTMPKRYDQDPANQGIVDALKADKKDPSGPYVWITYAAVQSLATALERTGSDEPLALVKDLKANGANTVIGPLNWDEKGDLKGFDFGVFQWHADGSSTAAK

SEQ ID NO: 3 - protein, 247 aa, Artificial Sequence
  cpYFP
MYNSDNVYIMADKQKNGIKANFKIRHNVEDGSVQLADHYQQNTPIGDGPVLLPDNHYLSFQSVLSKDPNEKRDHMVLLEFVTAAGITLGMDELYNVDGGSGGTGSKGEELFTGVVPILVELDGDVNGHKFSVSGEGEGDATYGKLTLKLICTTGKLPVPWPTLVTTLGYGLKCFARYPDHMKQHDFFKSAMPEGYVQERTIFFKDDGNYKTRAEVKFEGDTLVNRIELKGIGFKEDGNILGHKLEYN

SEQ ID NO: 4 - protein, 243 aa, Artificial Sequence
  cpBFP
NVYIKADKQKNGIKANFKIRHNIEGGGVQLAYHYQQNTPIGDGPVLLPDNHYLSVQSILSKDPNEKRDHMVLLEFVTAAGITLGMDELYKGGTGGSESMVSKGEELFTGVVPIQVELDGDVNGHKFSVSGEGEGDATYGKLTLKFICTTGKLPVPWPTLVTTLSHGVQCFSRYPDHMKQHDFFKSAMPGGYIQERTIFFKDDGNYKTRAEVKFEGDTLVNRIELKGIDFKEDGNILGHKLEYN

SEQ ID NO: 5 - protein, 243 aa, Artificial Sequence
  cpmApple
MVSERMYPEDGALKSEIKKGLRLKDGGHYAAEVKTTYKAKKPVQLPGAYIVDIKLDIVSHNEDYTIVEQCERAEGRHSTGGMDELYKGGTGGSLVSKGEEDNMAIIKEFMRFKVHMEGSVNGHEFEIEGEGEGRPYEAFQTAKLKVTKGGPLPFAWDILSPQFMYGSKAYIKHPADIPDYFKLSFPEGFRWERVMNFEDGGIIHVNQDSSLQDGVFIYKVKLRGTNFPPDGPVMQKKTMGWEA

SEQ ID NO: 6 - protein, 241 aa, Artificial Sequence
  cpGFP
NVYIKADKQKNGIKANFKIRHNIEDGGVQLAYHYQQNTPIGDGPVLLPDNHYLSVQSILSKDPNEKRDHMVLLEFVTAAGITLGMDELYKGGTGGSMVSKGEELFTGVVPIQVELDGDVNGHKFSVSGEGEGDATYGKLTLKFICTTGKLPVPWPTLVTTLTYGVQCFSRYPDHMKQHDFFKSAMPEGYIQERTIFFKDDGNYKTRAEVKFEGDTLVNRIELKGIDFKEDGNILGHKLEYN

SEQ ID NO: 7 - protein, 241 aa, Artificial Sequence
  cpTFP
NVYIMADKQKNGIKANFKIRHNIEDGGVQLADHYQQNTPIGDGPVLLPDNHYLSIQSKLSKDPNEKRDHMVLLEFVTAAGITHGMDELYKGGTGGSMVSKGEELFTGVVPILVELDGDVNGHKFSVSGEGEGDATYGKLTLKFICTTGKLPVPWPTLVTTFSYGVMVFARYPDHMKQHDFFKSAMPEGYVQERTIFFKDDGNYKTRAEVKFEGDTLVNRIELKGIDFKEDGNILGHKLEYN

SEQ ID NO: 8 - protein, 242 aa, Artificial Sequence
  cpmOrange
VSERMYPEDGVLKSEIKKGLRLKDGGHYAAEVKTTYKAKKPVQLPGAYIVDIKLDIVSHNEDYTIVEQCERAEGRHPTGGRDELYKGGTGGSLVSKGEEDNMAIIKEFMRFKVHMEGSVNGHEFEIEGEGEGRPYEAFQTAKLKVTKGGPLPFAWDILSPQFTYGSKAYIKHPADIPDYFKLSFPEGFRWERVMNFEDGGIIHVNQDSSLQDGVFIYKVKLRGTNFPPDGPVMQKKTMGWEA

SEQ ID NO: 9 - protein, 250 aa, Artificial Sequence
  cpmKate
MGGRSKKPAKNLKMPGVYYVDRRLERIKEADKETYVEQHEVAVARYCDLPSKLGHKLNGGTGGSMVSKGEELIKENMHMKLYMEGTVNNHHFKCTSEGEGKPYEGTQTMRIKVVEGGPLPFAFDILATSFMYGSKTFINHTQGIPDFFKQSFPEGFTWERVTTYEDGGVLTATQDTSLQDGCLIYNVKIRGVNFPSNGPVMQKKTLGWEASTEMLYPADGGLEGRSDMALKLVGGGHLICNLKTTYRSKK

SEQ ID NO: 10 - protein, 236 aa, Artificial Sequence
  mcherry
MVSKGEEDNMAIIKEFMRFKVHMEGSVNGHEFEIEGEGEGRPYEGTQTAKLKVTKGGPLPFAWDILSPQFMYGSKAYVKHPADIPDYLKLSFPEGFKWERVMNFEDGGVVTVTQDSSLQDGEFIYKVKLRGTNFPSDGPVMQKKTMGWEASSERMYPEDGALKGEIKQRLKLKDGGHYDAEVKTTYKAKKPVQLPGAYNVNIKLDITSHNEDYTIVEQYERAEGRHSTGGMDELYK

SEQ ID NO: 11 - protein, 238 aa, Artificial Sequence
  GFP
MSKGEELFTGVVPVLVELDGDVNGQKFSVSGEGEGDATYGKLTLNFICTTGKLPVPWPTLVTTFSYGVQCFSRYPDHMKQHDFFKSAMPEGYVQERTIFYKDDGNYKTRAEVKFEGDTLVNRIELKGIDFKEDGNILGHKMEYNYNSHNVYIMGDKPKNGIKVNFKIRHNIKDGSVQLADHYQQNTPIGDGPVLLPDNHYLSTQSALSKDPNEKRDHMILLEFVTAARITHGMDELYK

SEQ ID NO: 12 - protein, 239 aa, Artificial Sequence
  BFP
MVSKGEELFTGVVPILVELDGDVNGHKFSVSGEGEGDATYGKLTLKFICTTGKLPVPWPTLVTTLSHGVQCFSRYPDHMKQHDFFKSAMPEGYVQERTIFFKDDGNYKTRAEVKFEGDTLVNRIELKGIDFKEDGNILGHKLEYNFNSHNVYIMADKQKNGIKANFKIRHNIEDGSVQLADHYQQNTPIGDGPVLLPDSHYLSTQSALSKDPNEKRDHMVLLEFVTAAGITLGMDELYK

SEQ ID NO: 13 - protein, 233 aa, Artificial Sequence
  mKate
MSELITENMHMKLYMEGTVNNHHFKCTSEGEGKPYEGTQTMRIKVVEGGPLPFAFDILATSFMYGSKTFINHTQGIPDFFKQSFPEGFTWERVTTYEDGGVLTATQDTSLQDGCLIYNVKIRGVNFPSNGPVMQKKTLGWEASTEMLYPADGGLEGRADMALKLVGGGHLICNLKTTYRSKKPAKNLKMPGVYYVDRRLERIKEADKETYVEQHEVAVARYCDLPSKLGHKLN

SEQ ID NO: 14 - protein, 590 aa, Artificial Sequence
  LivJ325/326-cpYFP
EDIKVAVVGAMSGPVAQYGDQEFTGAEQAVADINAKGGIKGNKLQIVKYDDACDPKQAVAVANKVVNDGIKYVIGHLCSSSTQPASDIYEDEGILMITPAATAPELTARGYQLILRTTGLDSDQGPTAAKYILEKVKPQRIAIVHDKQQYGEGLARAVQDGLKKGNANVVFFDGITAGEKDFSTLVARLKKENIDFVYYGGYHPEMGQILRQARAAGLKTQFMGPEGVANVSLSNIAGESAEGLLVTKPKNYDQVPANKPIVDAIKAKKQDPSGAFVWTTYAALQSLQAGLNQSDDPAEIAKYLKANSVDTVMGPLTWDEKGDLKYNSDNVYIMADKQKNGIKANFKIRHNVEDGSVQLADHYQQNTPIGDGPVLLPDNHYLSFQSVLSKDPNEKRDHMVLLEFVTAAGITLGMDELYNVDGGSGGTGSKGEELFTGVVPILVELDGDVNGHKFSVSGEGEGDATYGKLTLKLICTTGKLPVPWPTLVTTLGYGLKCFARYPDHMKQHDFFKSAMPEGYVQERTIFFKDDGNYKTRAEVKFEGDTLVNRIELKGIGFKEDGNILGHKLEYNGFEFGVFDWHANGTATDAK

SEQ ID NO: 15 - protein, 589 aa, Artificial Sequence
  LivJ325/327-cpYFP
EDIKVAVVGAMSGPVAQYGDQEFTGAEQAVADINAKGGIKGNKLQIVKYDDACDPKQAVAVANKVVNDGIKYVIGHLCSSSTQPASDIYEDEGILMITPAATAPELTARGYQLILRTTGLDSDQGPTAAKYILEKVKPQRIAIVHDKQQYGEGLARAVQDGLKKGNANVVFFDGITAGEKDFSTLVARLKKENIDFVYYGGYHPEMGQILRQARAAGLKTQFMGPEGVANVSLSNIAGESAEGLLVTKPKNYDQVPANKPIVDAIKAKKQDPSGAFVWTTYAALQSLQAGLNQSDDPAEIAKYLKANSVDTVMGPLTWDEKGDLKYNSDNVYIMADKQKNGIKANFKIRHNVEDGSVQLADHYQQNTPIGDGPVLLPDNHYLSFQSVLSKDPNEKRDHMVLLEFVTAAGITLGMDELYNVDGGSGGTGSKGEELFTGVVPILVELDGDVNGHKFSVSGEGEGDATYGKLTLKLICTTGKLPVPWPTLVTTLGYGLKCFARYPDHMKQHDFFKSAMPEGYVQERTIFFKDDGNYKTRAEVKFEGDTLVNRIELKGIGFKEDGNILGHKLEYNFEFGVFDWHANGTATDAK

SEQ ID NO: 16 - protein, 588 aa, Artificial Sequence
  LivJ325/328-cpYFP
EDIKVAVVGAMSGPVAQYGDQEFTGAEQAVADINAKGGIKGNKLQIVKYDDACDPKQAVAVANKVVNDGIKYVIGHLCSSSTQPASDIYEDEGILMITPAATAPELTARGYQLILRTTGLDSDQGPTAAKYILEKVKPQRIAIVHDKQQYGEGLARAVQDGLKKGNANVVFFDGITAGEKDFSTLVARLKKENIDFVYYGGYHPEMGQILRQARAAGLKTQFMGPEGVANVSLSNIAGESAEGLLVTKPKNYDQVPANKPIVDAIKAKKQDPSGAFVWTTYAALQSLQAGLNQSDDPAEIAKYLKANSVDTVMGPLTWDEKGDLKYNSDNVYIMADKQKNGIKANFKIRHNVEDGSVQLADHYQQNTPIGDGPVLLPDNHYLSFQSVLSKDPNEKRDHMVLLEFVTAAGITLGMDELYNVDGGSGGTGSKGEELFTGVVPILVELDGDVNGHKFSVSGEGEGDATYGKLTLKLICTTGKLPVPWPTLVTTLGYGLKCFARYPDHMKQHDFFKSAMPEGYVQERTIFFKDDGNYKTRAEVKFEGDTLVNRIELKGIGFKEDGNILGHKLEYNEFGVFDWHANGTATDAK

SEQ ID NO: 17 - protein, 587 aa, Artificial Sequence
  LivJ325/329-cpYFP
EDIKVAVVGAMSGPVAQYGDQEFTGAEQAVADINAKGGIKGNKLQIVKYDDACDPKQAVAVANKVVNDGIKYVIGHLCSSSTQPASDIYEDEGILMITPAATAPELTARGYQLILRTTGLDSDQGPTAAKYILEKVKPQRIAIVHDKQQYGEGLARAVQDGLKKGNANVVFFDGITAGEKDFSTLVARLKKENIDFVYYGGYHPEMGQILRQARAAGLKTQFMGPEGVANVSLSNIAGESAEGLLVTKPKNYDQVPANKPIVDAIKAKKQDPSGAFVWTTYAALQSLQAGLNQSDDPAEIAKYLKANSVDTVMGPLTWDEKGDLKYNSDNVYIMADKQKNGIKANFKIRHNVEDGSVQLADHYQQNTPIGDGPVLLPDNHYLSFQSVLSKDPNEKRDHMVLLEFVTAAGITLGMDELYNVDGGSGGTGSKGEELFTGVVPILVELDGDVNGHKFSVSGEGEGDATYGKLTLKLICTTGKLPVPWPTLVTTLGYGLKCFARYPDHMKQHDFFKSAMPEGYVQERTIFFKDDGNYKTRAEVKFEGDTLVNRIELKGIGFKEDGNILGHKLEYNFGVFDWHANGTATDAK

SEQ ID NO: 18 - protein, 591 aa, Artificial Sequence
  LivJ326/327-cpYFP
MEDIKVAVVGAMSGPVAQYGDQEFTGAEQAVADINAKGGIKGNKLQIVKYDDACDPKQAVAVANKVVNDGIKYVIGHLCSSSTQPASDIYEDEGILMITPAATAPELTARGYQLILRTTGLDSDQGPTAAKYILEKVKPQRIAIVHDKQQYGEGLARAVQDGLKKGNANVVFFDGITAGEKDFSTLVARLKKENIDFVYYGGYHPEMGQILRQARAAGLKTQFMGPEGVANVSLSNIAGESAEGLLVTKPKNYDQVPANKPIVDAIKAKKQDPSGAFVWTTYAALQSLQAGLNQSDDPAEIAKYLKANSVDTVMGPLTWDEKGDLKGYNSDNVYIMADKQKNGIKANFKIRHNVEDGSVQLADHYQQNTPIGDGPVLLPDNHYLSFQSVLSKDPNEKRDHMVLLEFVTAAGITLGMDELYNVDGGSGGTGSKGEELFTGVVPILVELDGDVNGHKFSVSGEGEGDATYGKLTLKLICTTGKLPVPWPTLVTTLGYGLKCFARYPDHMKQHDFFKSAMPEGYVQERTIFFKDDGNYKTRAEVKFEGDTLVNRIELKGIGFKEDGNILGHKLEYNFEFGVFDWHANGTATDAK

SEQ ID NO: 19 - protein, 589 aa, Artificial Sequence
  LivJ326/328-cpYFP
EDIKVAVVGAMSGPVAQYGDQEFTGAEQAVADINAKGGIKGNKLQIVKYDDACDPKQAVAVANKVVNDGIKYVIGHLCSSSTQPASDIYEDEGILMITPAATAPELTARGYQLILRTTGLDSDQGPTAAKYILEKVKPQRIAIVHDKQQYGEGLARAVQDGLKKGNANVVFFDGITAGEKDFSTLVARLKKENIDFVYYGGYHPEMGQILRQARAAGLKTQFMGPEGVANVSLSNIAGESAEGLLVTKPKNYDQVPANKPIVDAIKAKKQDPSGAFVWTTYAALQSLQAGLNQSDDPAEIAKYLKANSVDTVMGPLTWDEKGDLKGYNSDNVYIMADKQKNGIKANFKIRHNVEDGSVQLADHYQQNTPIGDGPVLLPDNHYLSFQSVLSKDPNEKRDHMVLLEFVTAAGITLGMDELYNVDGGSGGTGSKGEELFTGVVPILVELDGDVNGHKFSVSGEGEGDATYGKLTLKLICTTGKLPVPWPTLVTTLGYGLKCFARYPDHMKQHDFFKSAMPEGYVQERTIFFKDDGNYKTRAEVKFEGDTLVNRIELKGIGFKEDGNILGHKLEYNEFGVFDWHANGTATDAK

SEQ ID NO: 20 - protein, 588 aa, Artificial Sequence
  LivJ326/329-cpYFP
EDIKVAVVGAMSGPVAQYGDQEFTGAEQAVADINAKGGIKGNKLQIVKYDDACDPKQAVAVANKVVNDGIKYVIGHLCSSSTQPASDIYEDEGILMITPAATAPELTARGYQLILRTTGLDSDQGPTAAKYILEKVKPQRIAIVHDKQQYGEGLARAVQDGLKKGNANVVFFDGITAGEKDFSTLVARLKKENIDFVYYGGYHPEMGQILRQARAAGLKTQFMGPEGVANVSLSNIAGESAEGLLVTKPKNYDQVPANKPIVDAIKAKKQDPSGAFVWTTYAALQSLQAGLNQSDDPAEIAKYLKANSVDTVMGPLTWDEKGDLKGYNSDNVYIMADKQKNGIKANFKIRHNVEDGSVQLADHYQQNTPIGDGPVLLPDNHYLSFQSVLSKDPNEKRDHMVLLEFVTAAGITLGMDELYNVDGGSGGTGSKGEELFTGVVPILVELDGDVNGHKFSVSGEGEGDATYGKLTLKLICTTGKLPVPWPTLVTTLGYGLKCFARYPDHMKQHDFFKSAMPEGYVQERTIFFKDDGNYKTRAEVKFEGDTLVNRIELKGIGFKEDGNILGHKLEYNFGVFDWHANGTATDAK

SEQ ID NO: 21 - protein, 591 aa, Artificial Sequence
  LivJ327/328-cpYFP
MEDIKVAVVGAMSGPVAQYGDQEFTGAEQAVADINAKGGIKGNKLQIVKYDDACDPKQAVAVANKVVNDGIKYVIGHLCSSSTQPASDIYEDEGILMITPAATAPELTARGYQLILRTTGLDSDQGPTAAKYILEKVKPQRIAIVHDKQQYGEGLARAVQDGLKKGNANVVFFDGITAGEKDFSTLVARLKKENIDFVYYGGYHPEMGQILRQARAAGLKTQFMGPEGVANVSLSNIAGESAEGLLVTKPKNYDQVPANKPIVDAIKAKKQDPSGAFVWTTYAALQSLQAGLNQSDDPAEIAKYLKANSVDTVMGPLTWDEKGDLKGFYNSDNVYIMADKQKNGIKANFKIRHNVEDGSVQLADHYQQNTPIGDGPVLLPDNHYLSFQSVLSKDPNEKRDHMVLLEFVTAAGITLGMDELYNVDGGSGGTGSKGEELFTGVVPILVELDGDVNGHKFSVSGEGEGDATYGKLTLKLICTTGKLPVPWPTLVTTLGYGLKCFARYPDHMKQHDFFKSAMPEGYVQERTIFFKDDGNYKTRAEVKFEGDTLVNRIELKGIGFKEDGNILGHKLEYNEFGVFDWHANGTATDAK

SEQ ID NO: 22 - protein, 589 aa, Artificial Sequence
  LivJ327/329-cpYFP
EDIKVAVVGAMSGPVAQYGDQEFTGAEQAVADINAKGGIKGNKLQIVKYDDACDPKQAVAVANKVVNDGIKYVIGHLCSSSTQPASDIYEDEGILMITPAATAPELTARGYQLILRTTGLDSDQGPTAAKYILEKVKPQRIAIVHDKQQYGEGLARAVQDGLKKGNANVVFFDGITAGEKDFSTLVARLKKENIDFVYYGGYHPEMGQILRQARAAGLKTQFMGPEGVANVSLSNIAGESAEGLLVTKPKNYDQVPANKPIVDAIKAKKQDPSGAFVWTTYAALQSLQAGLNQSDDPAEIAKYLKANSVDTVMGPLTWDEKGDLKGFYNSDNVYIMADKQKNGIKANFKIRHNVEDGSVQLADHYQQNTPIGDGPVLLPDNHYLSFQSVLSKDPNEKRDHMVLLEFVTAAGITLGMDELYNVDGGSGGTGSKGEELFTGVVPILVELDGDVNGHKFSVSGEGEGDATYGKLTLKLICTTGKLPVPWPTLVTTLGYGLKCFARYPDHMKQHDFFKSAMPEGYVQERTIFFKDDGNYKTRAEVKFEGDTLVNRIELKGIGFKEDGNILGHKLEYNFGVFDWHANGTATDAK

SEQ ID NO: 23 - protein, 590 aa, Artificial Sequence
  LivJ328/329-cpYFP
EDIKVAVVGAMSGPVAQYGDQEFTGAEQAVADINAKGGIKGNKLQIVKYDDACDPKQAVAVANKVVNDGIKYVIGHLCSSSTQPASDIYEDEGILMITPAATAPELTARGYQLILRTTGLDSDQGPTAAKYILEKVKPQRIAIVHDKQQYGEGLARAVQDGLKKGNANVVFFDGITAGEKDFSTLVARLKKENIDFVYYGGYHPEMGQILRQARAAGLKTQFMGPEGVANVSLSNIAGESAEGLLVTKPKNYDQVPANKPIVDAIKAKKQDPSGAFVWTTYAALQSLQAGLNQSDDPAEIAKYLKANSVDTVMGPLTWDEKGDLKGFEYNSDNVYIMADKQKNGIKANFKIRHNVEDGSVQLADHYQQNTPIGDGPVLLPDNHYLSFQSVLSKDPNEKRDHMVLLEFVTAAGITLGMDELYNVDGGSGGTGSKGEELFTGVVPILVELDGDVNGHKFSVSGEGEGDATYGKLTLKLICTTGKLPVPWPTLVTTLGYGLKCFARYPDHMKQHDFFKSAMPEGYVQERTIFFKDDGNYKTRAEVKFEGDTLVNRIELKGIGFKEDGNILGHKLEYNFGVFDWHANGTATDAK

SEQ ID NO: 24 - protein, 593 aa, Artificial Sequence
  LivK 327/328-cpYFP
MDDIKVAVVGAMSGPIAQWGDMEFNGARQAIKDINAKGGIKGDKLVGVEYDDACDPKQAVAVANKIVNDGIKYVIGHLCSSSTQPASDIYEDEGILMISPGATNPELTQRGYQHIMRTAGLDSSQGPTAAKYILETVKPQRIAIIHDKQQYGEGLARSVQDGLKAANANVVFFDGITAGEKDFSALIARLKKENIDFVYYGGYYPEMGQMLRQARSVGLKTQFMGPEGVGNASLSNIAGDAAEGMLVTMPKRYDQDPANQGIVDALKADKKDPSGPYVWITYAAVQSLATALERTGSDEPLALVKDLKANGANTVIGPLNWDEKGDLKYNSDNVYIMADKQKNGIKANFKIRHNVEDGSVQLADHYQQNTPIGDGPVLLPDNHYLSFQSVLSKDPNEKRDHMVLLEFVTAAGITLGMDELYNVDGGSGGTGSKGEELFTGVVPILVELDGDVNGHKFSVSGEGEGDATYGKLTLKLICTTGKLPVPWPTLVTTLGYGLKCFARYPDHMKQHDFFKSAMPEGYVQERTIFFKDDGNYKTRAEVKFEGDTLVNRIELKGIGFKEDGNILGHKLEYNGFDFGVFQWHADGSSTAAK

SEQ ID NO: 25 - protein, 592 aa, Artificial Sequence
  LivK 327/329-cpYFP
MDDIKVAVVGAMSGPIAQWGDMEFNGARQAIKDINAKGGIKGDKLVGVEYDDACDPKQAVAVANKIVNDGIKYVIGHLCSSSTQPASDIYEDEGILMISPGATNPELTQRGYQHIMRTAGLDSSQGPTAAKYILETVKPQRIAIIHDKQQYGEGLARSVQDGLKAANANVVFFDGITAGEKDFSALIARLKKENIDFVYYGGYYPEMGQMLRQARSVGLKTQFMGPEGVGNASLSNIAGDAAEGMLVTMPKRYDQDPANQGIVDALKADKKDPSGPYVWITYAAVQSLATALERTGSDEPLALVKDLKANGANTVIGPLNWDEKGDLKYNSDNVYIMADKQKNGIKANFKIRHNVEDGSVQLADHYQQNTPIGDGPVLLPDNHYLSFQSVLSKDPNEKRDHMVLLEFVTAAGITLGMDELYNVDGGSGGTGSKGEELFTGVVPILVELDGDVNGHKFSVSGEGEGDATYGKLTLKLICTTGKLPVPWPTLVTTLGYGLKCFARYPDHMKQHDFFKSAMPEGYVQERTIFFKDDGNYKTRAEVKFEGDTLVNRIELKGIGFKEDGNILGHKLEYNFDFGVFQWHADGSSTAAK

SEQ ID NO: 26 - protein, 591 aa, Artificial Sequence
  LivK 327/330-cpYFP
MDDIKVAVVGAMSGPIAQWGDMEFNGARQAIKDINAKGGIKGDKLVGVEYDDACDPKQAVAVANKIVNDGIKYVIGHLCSSSTQPASDIYEDEGILMISPGATNPELTQRGYQHIMRTAGLDSSQGPTAAKYILETVKPQRIAIIHDKQQYGEGLARSVQDGLKAANANVVFFDGITAGEKDFSALIARLKKENIDFVYYGGYYPEMGQMLRQARSVGLKTQFMGPEGVGNASLSNIAGDAAEGMLVTMPKRYDQDPANQGIVDALKADKKDPSGPYVWITYAAVQSLATALERTGSDEPLALVKDLKANGANTVIGPLNWDEKGDLKYNSDNVYIMADKQKNGIKANFKIRHNVEDGSVQLADHYQQNTPIGDGPVLLPDNHYLSFQSVLSKDPNEKRDHMVLLEFVTAAGITLGMDELYNVDGGSGGTGSKGEELFTGVVPILVELDGDVNGHKFSVSGEGEGDATYGKLTLKLICTTGKLPVPWPTLVTTLGYGLKCFARYPDHMKQHDFFKSAMPEGYVQERTIFFKDDGNYKTRAEVKFEGDTLVNRIELKGIGFKEDGNILGHKLEYNDFGVFQWHADGSSTAAK

SEQ ID NO: 27 - protein, 593 aa, Artificial Sequence; identical to SEQ ID NO: 24
  LivK 327/331-cpYFP

SEQ ID NO: 28 - protein, 593 aa, Artificial Sequence
  LivK 328/329-cpYFP
MDDIKVAVVGAMSGPIAQWGDMEFNGARQAIKDINAKGGIKGDKLVGVEYDDACDPKQAVAVANKIVNDGIKYVIGHLCSSSTQPASDIYEDEGILMISPGATNPELTQRGYQHIMRTAGLDSSQGPTAAKYILETVKPQRIAIIHDKQQYGEGLARSVQDGLKAANANVVFFDGITAGEKDFSALIARLKKENIDFVYYGGYYPEMGQMLRQARSVGLKTQFMGPEGVGNASLSNIAGDAAEGMLVTMPKRYDQDPANQGIVDALKADKKDPSGPYVWITYAAVQSLATALERTGSDEPLALVKDLKANGANTVIGPLNWDEKGDLKGYNSDNVYIMADKQKNGIKANFKIRHNVEDGSVQLADHYQQNTPIGDGPVLLPDNHYLSFQSVLSKDPNEKRDHMVLLEFVTAAGITLGMDELYNVDGGSGGTGSKGEELFTGVVPILVELDGDVNGHKFSVSGEGEGDATYGKLTLKLICTTGKLPVPWPTLVTTLGYGLKCFARYPDHMKQHDFFKSAMPEGYVQERTIFFKDDGNYKTRAEVKFEGDTLVNRIELKGIGFKEDGNILGHKLEYNFDFGVFQWHADGSSTAAK

SEQ ID NO: 29 - protein, 593 aa, Artificial Sequence; identical to SEQ ID NO: 28
  LivK 328/330-cpYFP

SEQ ID NO: 30 - protein, 593 aa, Artificial Sequence; identical to SEQ ID NO: 28
  LivK 328/331-cpYFP

SEQ ID NO: 31 - protein, 593 aa, Artificial Sequence
  LivK 329/330-cpYFP
MDDIKVAVVGAMSGPIAQWGDMEFNGARQAIKDINAKGGIKGDKLVGVEYDDACDPKQAVAVANKIVNDGIKYVIGHLCSSSTQPASDIYEDEGILMISPGATNPELTQRGYQHIMRTAGLDSSQGPTAAKYILETVKPQRIAIIHDKQQYGEGLARSVQDGLKAANANVVFFDGITAGEKDFSALIARLKKENIDFVYYGGYYPEMGQMLRQARSVGLKTQFMGPEGVGNASLSNIAGDAAEGMLVTMPKRYDQDPANQGIVDALKADKKDPSGPYVWITYAAVQSLATALERTGSDEPLALVKDLKANGANTVIGPLNWDEKGDLKGFYNSDNVYIMADKQKNGIKANFKIRHNVEDGSVQLADHYQQNTPIGDGPVLLPDNHYLSFQSVLSKDPNEKRDHMVLLEFVTAAGITLGMDELYNVDGGSGGTGSKGEELFTGVVPILVELDGDVNGHKFSVSGEGEGDATYGKLTLKLICTTGKLPVPWPTLVTTLGYGLKCFARYPDHMKQHDFFKSAMPEGYVQERTIFFKDDGNYKTRAEVKFEGDTLVNRIELKGIGFKEDGNILGHKLEYNDFGVFQWHADGSSTAAK

SEQ ID NO: 32 - protein, 593 aa, Artificial Sequence; identical to SEQ ID NO: 31
  LivK 329/331-cpYFP

SEQ ID NO: 33 - protein, 593 aa, Artificial Sequence
  LivK 330/331-cpYFP
MDDIKVAVVGAMSGPIAQWGDMEFNGARQAIKDINAKGGIKGDKLVGVEYDDACDPKQAVAVANKIVNDGIKYVIGHLCSSSTQPASDIYEDEGILMISPGATNPELTQRGYQHIMRTAGLDSSQGPTAAKYILETVKPQRIAIIHDKQQYGEGLARSVQDGLKAANANVVFFDGITAGEKDFSALIARLKKENIDFVYYGGYYPEMGQMLRQARSVGLKTQFMGPEGVGNASLSNIAGDAAEGMLVTMPKRYDQDPANQGIVDALKADKKDPSGPYVWITYAAVQSLATALERTGSDEPLALVKDLKANGANTVIGPLNWDEKGDLKGFDYNSDNVYIMADKQKNGIKANFKIRHNVEDGSVQLADHYQQNTPIGDGPVLLPDNHYLSFQSVLSKDPNEKRDHMVLLEFVTAAGITLGMDELYNVDGGSGGTGSKGEELFTGVVPILVELDGDVNGHKFSVSGEGEGDATYGKLTLKLICTTGKLPVPWPTLVTTLGYGLKCFARYPDHMKQHDFFKSAMPEGYVQERTIFFKDDGNYKTRAEVKFEGDTLVNRIELKGIGFKEDGNILGHKLEYNFGVFQWHADGSSTAAK